European Patent Specification EP 3 561 057 B1, published July 23, 2025. Title: Anti-CD3 Antibody and Molecule comprising the Antibody thereof. Applicant: DAIICHI SANKYO COMPANY, LIMITED. The sequence listing filed with the application follows.

SEQUENCE LISTING (103 sequences)

SEQ ID NO: 1 - protein, 207 aa, Homo sapiens
MQSGTHWRVLGLCLLSVGVWGQDGNEEMGGITQTPYKVSISGTTVILTCPQYPGSEILWQHNDKNIGGDEDDKNIGSDEDHLSLKEFSELEQSGYYVCYPRGSKPEDANFYLYLRARVCENCMEMDVMSVATIVIVDICITGGLLLLVYYWSKNRKAKAKPVTRGAGAGGRQRGQNKERPPPVPNPDYEPIRKGQRDLYSGLNQRRI

SEQ ID NO: 2 - protein, 171 aa, Homo sapiens
MEHSTFLSGLVLATLLSQVSPFKIPIEELEDRVFVNCNTSITWVEGTVGTLLSDITRLDLGKRILDPRGIYRCNGTDIYKDKESTVQVHYRMCQSCVELDPATVAGIIVTDVIATLLLALGVFCFAGHETGRLSGAADTQALLRNDQVYQPLRDRDDAQYSHLGGNWARNK

SEQ ID NO: 3 - protein, 182 aa, Homo sapiens
MEQGKGLAVLILAIILLQGTLAQSIKGNHLVKVYDYQEDGSVLLTCDAEAKNITWFKDGKMIGFLTEDKKKWNLGSNAKDPRGMYQCKGSQNKSKPLQVYYRMCQNCIELNAATISGFLFAEIVSIFVLAVGVYFIAGQDGVRQSRASDKQTLLPNDQLYQPLKDREDDQYSHLQGNQLRRN

SEQ ID NO: 4 - DNA, 657 bp, Artificial Sequence
  CD3 epsilon gamma DNA
atgagaggatcgcatcaccatcaccatcacggatcccagagcattaaaggtaatcacctggtgaaagtgtatgactatcaagaagatggtagcgttctgctgacctgtgatgcagaagcaaaaaacattacctggttcaaagacggcaaaatgattggttttctgaccgaagataaaaaaaaatggaatctgggcagcaatgcaaaagatccgcgtggtatgtatcagtgtaaaggtagccagaataaaagcaaaccgctgcaggtttattatcgtatgggtagcgcagatgatgcaaaaaaagatgcagccaaaaaagacgacgcgaaaaaagatgatgctaaaaaagacggttccgatggcaatgaagaaatgggtggtattacccagaccccgtataaagttagcattagcggcaccaccgttattctgacctgtccgcagtatccgggtagcgaaattctgtggcagcataacgataaaaacattggcggtgatgaggacgacaaaaatatcggtagtgatgaagatcatctgagcctgaaagaattcagcgaactggaacagagcggttattatgtttgttatcctcgtggtagcaaaccggaagatgcaaacttttatctgtatctgcgtgcacgtgttgggaagcttaat

SEQ ID NO: 5 - protein, 219 aa, Artificial Sequence
  His-scCD3 AA
MRGSHHHHHHGSQSIKGNHLVKVYDYQEDGSVLLTCDAEAKNITWFKDGKMIGFLTEDKKKWNLGSNAKDPRGMYQCKGSQNKSKPLQVYYRMGSADDAKKDAAKKDDAKKDDAKKDGSDGNEEMGGITQTPYKVSISGTTVILTCPQYPGSEILWQHNDKNIGGDEDDKNIGSDEDHLSLKEFSELEQSGYYVCYPRGSKPEDANFYLYLRARVGKLN

SEQ ID NO: 6 - DNA, 354 bp, Rutilus rutilus
gaggtgcagttggtggagtctgggggaggcctggtgcagcctggaagggccctgaaactctcctgtgtagtctctggagtcacattcaattactacgggatgagctggatccgccaggctccagggaaggggctggagtgggttgcatccattactaattctggtggtagaatttactatccagactctgtgaagggccgattcactatctccagagaaaatacacaaaagaccctatacctacaaatgaacagtctgaggtctgaggacacggccacttattactgtactctcgatggtcgcgatggttgggttgcttactggggccaaggcactctggtcactgtctcttca

SEQ ID NO: 7 - protein, 118 aa, Rutilus rutilus
EVQLVESGGGLVQPGRALKLSCVVSGVTFNYYGMSWIRQAPGKGLEWVASITNSGGRIYYPDSVKGRFTISRENTQKTLYLQMNSLRSEDTATYYCTLDGRDGWVAYWGQGTLVTVSS

SEQ ID NO: 8 - DNA, 327 bp, Rutilus rutilus
cagtttgtgcttactcagccaaactctgtgtctacgaatctcggaaccacagtcgaactgtcttgcaagcgcaacactgggaacattggaagcaattatgtgaactggtaccagcagcatgagggaagatctcccaccactattatttatagggatgataagagaccagatggagtttctgacaggttctctgggtccattgacagatcttccaagtcagccctcctgacaatcaataatgtgcagactgaagatgaagctgactacttctgtcagtcttacagtagtggttttattttcggcggtggaaccaagctcactgtccta

SEQ ID NO: 9 - protein, 109 aa, Artificial Sequence
  C3-147_VL AA
QFVLTQPNSVSTNLGTTVELSCKRNTGNIGSNYVNWYQQHEGRSPTTIIYRDDKRPDGVSDRFSGSIDRSSKSALLTINNVQTEDEADYFCQSYSSGFIFGGGTKLTVL

SEQ ID NO: 10 - DNA, 75 bp, Artificial Sequence
  G4S linker sense
gtcactgtctcttcaggtggaggcggttcaggcggaggtggcagcggcggtggcgggagtcagtttgtgcttact

SEQ ID NO: 11 - DNA, 75 bp, Artificial Sequence
  G4sS linker antisense
agtaagcacaaactgactcccgccaccgccgctgccacctccgcctgaaccgcctccacctgaagagacagtgac

SEQ ID NO: 12 - protein, 118 aa, Rutilus rutilus; identical to SEQ ID NO: 7

SEQ ID NO: 13 - protein, 109 aa, Rutilus rutilus; identical to SEQ ID NO: 9

SEQ ID NO: 14 - DNA, 867 bp, Artificial Sequence
  C3E-7000 ORF
atgaaacacctgtggttcttcctcctgctggtggcagctcccagatgggtgctgagcgaggtgcagttggtggagtctgggggaggcctggtgcagcctggaagggccctgaaactctcctgtgtagtctctggagtcacattcaattactacgggatgagctggatccgccaggctccagggaaggggctggagtgggttgcatccattactaattctggtggtagaatttactatccagactctgtgaagggccgattcactatctccagagaaaatacacaaaagaccctatacctacaaatgaacagtctgaggtctgaggacacggccacttattactgtactctcgatggtcgcgatggttgggttgcttactggggccaaggcactctggtcactgtctcttcaggtggaggcggttcaggcggaggtggcagcggcggtggcgggagtcagtttgtgcttactcagccaaactctgtgtctacgaatctcggaaccacagtcgaactgtcttgcaagcgcaacactgggaacattggaagcaattatgtgaactggtaccagcagcatgagggaagatctcccaccactattatttatagggatgataagagaccagatggagtttctgacaggttctctgggtccattgacagatcttccaagtcagccctcctgacaatcaataatgtgcagactgaagatgaagctgactacttctgtcagtcttacagtagtggttttattttcggcggtggaaccaagctcactgtcctaggcgcgtctgcggccgcaggatccggtggtgattacaaagatgatgacgataaaggtgcagcggcgcatcaccatcatcaccac

SEQ ID NO: 15 - protein, 270 aa, Artificial Sequence
  C3E-7000 AA
EVQLVESGGGLVQPGRALKLSCVVSGVTFNYYGMSWIRQAPGKGLEWVASITNSGGRIYYPDSVKGRFTISRENTQKTLYLQMNSLRSEDTATYYCTLDGRDGWVAYWGQGTLVTVSSGGGGSGGGGSGGGGSQFVLTQPNSVSTNLGTTVELSCKRNTGNIGSNYVNWYQQHEGRSPTTIIYRDDKRPDGVSDRFSGSIDRSSKSALLTINNVQTEDEADYFCQSYSSGFIFGGGTKLTVLGASAAAGSGGDYKDDDDKGAAAHHHHHH

SEQ ID NO: 16 - protein, 118 aa, Artificial Sequence
  C3E-7034_VH AA
EVQLVESGGGLVQPGGSLRLSCAASGVTFNYYGMSWIRQAPGKGLEWVASITNSGGRIYYPDSVKGRFTISRENTQKTLYLQMNSLRAEDTAVYYCTLDGRDGWVAYWGQGTLVTVSS

SEQ ID NO: 17 - protein, 109 aa, Artificial Sequence
  C3E-7034_VL AA
NFMLTQPHSVSESPGKTVTISCKRNTGNIGSNYVNWYQQHEGSSPTTIIYRDDKRPDGVSDRFSGSIDRSSKSASLTISNLKTEDEADYFCQSYSSGFIFGGGTKLTVL

SEQ ID NO: 18 - DNA, 864 bp, Artificial Sequence
  C3E-7034 ORF
atgaaacacctgtggttcttcctcctgctggtggcagctcccagatgggtgctgagcggagaagtgcagctggtggaatccggggggggcctggtgcagcctggggggagcctgagactgagttgtgccgcctctggggtgacatttaactactatggcatgtcttggatccgccaggcacctggaaagggcctggagtgggtggccagcatcactaattccggcgggcgaatctactatcccgacagcgtcaagggcaggttcacaatttcccgcgagaacacacagaaaactctgtacctgcagatgaatagcctgagagccgaagatacagctgtgtactattgcactctggacggcagggatgggtgggtcgcctattgggggcagggaaccctggtgacagtcagctccggaggaggaggatctggcggaggaggcagtgggggaggcgggtcaaactttatgctgacccagccccacagtgtgtcagagagccctggcaagactgtcaccatctcttgtaaaaggaacaccggaaatattggcagtaactacgtgaattggtatcagcagcatgaagggtctagtccaaccacaatcatctaccgggacgataagagacccgacggggtgtccgatcgattctccggatctatcgaccggtcaagcaagagtgcttcactgaccattagcaatctgaaaacagaggacgaagcagattacttttgccagtcctattcctctggcttcatctttggaggcgggactaaactgaccgtgctgggcgcggccgcaggtgcaggtggtgattacaaagatgatgacgataaaggtgcagcggcgcatcaccatcatcaccac

SEQ ID NO: 19 - protein, 269 aa, Artificial Sequence
  C3E-7034 AA
GEVQLVESGGGLVQPGGSLRLSCAASGVTFNYYGMSWIRQAPGKGLEWVASITNSGGRIYYPDSVKGRFTISRENTQKTLYLQMNSLRAEDTAVYYCTLDGRDGWVAYWGQGTLVTVSSGGGGSGGGGSGGGGSNFMLTQPHSVSESPGKTVTISCKRNTGNIGSNYVNWYQQHEGSSPTTIIYRDDKRPDGVSDRFSGSIDRSSKSASLTISNLKTEDEADYFCQSYSSGFIFGGGTKLTVLGAAAGAGGDYKDDDDKGAAAHHHHHH

SEQ ID NO: 20 - protein, 107 aa, Artificial Sequence
  C3E-7035_VL AA
QAVLTQPSSVSGVPGQRVTISCKRNTGNIGSNYVNWYQQLPGTAPKLLIYRDDKRPSGVPDRFSGSKSGTSASLAITGFQAEDEADYYCQSYSSGFIFGGGTKLTVL

SEQ ID NO: 21 - DNA, 864 bp, Artificial Sequence
  C3E-7035 ORF
atgaaacacctgtggttcttcctcctgctggtggcagctcccagatgggtgctgagcggagaagtgcagctggtggaatccggggggggcctggtgcagcctggggggagcctgagactgagttgtgccgcctctggggtgacatttaactactatggcatgtcttggatccgccaggcacctggaaagggcctggagtgggtggccagcatcactaattccggcgggcgaatctactatcccgacagcgtcaagggcaggttcacaatttcccgcgagaacacacagaaaactctgtacctgcagatgaatagcctgagagccgaagatacagctgtgtactattgcactctggacggcagggatgggtgggtcgcctattgggggcagggaaccctggtgacagtcagctccggaggaggaggatctggcggaggaggcagtgggggaggcgggtcaatggcccaggctgtgctcactcagccgtcctctgtttctggcgtacctggccaacgggtgaccattagctgtaaaaggaataccgggaatatcgggtctaactacgtgaactggtatcagcagcttccagggacagctcccaagttgctgatctatcgcgacgacaaaagaccctcaggggtccctgaccgatttagtggcagcaaaagcggtacttccgcttccctggcgataaccggctttcaggccgaagatgaggcagactactattgccagtcatattccagcggcttcatcttcggaggcggaactaagctgacagtgctgggcgcggccgcaggtgcaggtggtgattacaaagatgatgacgataaaggtgcagcggcgcatcaccatcatcaccac

SEQ ID NO: 22 - protein, 269 aa, Artificial Sequence
  C3E-7035 AA
GEVQLVESGGGLVQPGGSLRLSCAASGVTFNYYGMSWIRQAPGKGLEWVASITNSGGRIYYPDSVKGRFTISRENTQKTLYLQMNSLRAEDTAVYYCTLDGRDGWVAYWGQGTLVTVSSGGGGSGGGGSGGGGSMAQAVLTQPSSVSGVPGQRVTISCKRNTGNIGSNYVNWYQQLPGTAPKLLIYRDDKRPSGVPDRFSGSKSGTSASLAITGFQAEDEADYYCQSYSSGFIFGGGTKLTVLGAAAGAGGDYKDDDDKGAAAHHHHHH

SEQ ID NO: 23 - protein, 107 aa, Artificial Sequence
  C3E-7036_VL AA
NFMLTQPSSVSGVPGQRVTISCTGNTGNIGSNYVNWYQQLPGTAPKLLIYRDDKRPSGVPDRFSGSKSGTSASLAITGFQAEDEADYYCQSYSSGFIFGGGTKLTVL

SEQ ID NO: 24 - DNA, 858 bp, Artificial Sequence
  C3E-7036 ORF
atgaaacacctgtggttcttcctcctgctggtggcagctcccagatgggtgctgagcggagaagtgcagctggtggaatccggggggggcctggtgcagcctggggggagcctgagactgagttgtgccgcctctggggtgacatttaactactatggcatgtcttggatccgccaggcacctggaaagggcctggagtgggtggccagcatcactaattccggcgggcgaatctactatcccgacagcgtcaagggcaggttcacaatttcccgcgagaacacacagaaaactctgtacctgcagatgaatagcctgagagccgaagatacagctgtgtactattgcactctggacggcagggatgggtgggtcgcctattgggggcagggaaccctggtgacagtcagctccggaggaggaggatctggcggaggaggcagtgggggaggcgggtcaaactttatgctcactcagccgtcctctgtttctggcgtacctggccaacgggtgaccattagctgtacgggtaataccgggaatatcgggtctaactacgtgaactggtatcagcagcttccagggacagctcccaagttgctgatctatcgcgacgacaaaagaccctcaggggtccctgaccgatttagtggcagcaaaagcggtacttccgcttccctggcgataaccggctttcaggccgaagatgaggcagactactattgccagtcatattccagcggcttcatcttcggaggcggaactaagctgacagtgttgggtgcggccgcaggtgcaggtggtgattacaaagatgatgacgataaaggtgcagcggcgcatcaccatcatcaccac

SEQ ID NO: 25 - protein, 267 aa, Artificial Sequence
  C3E-7036 AA
GEVQLVESGGGLVQPGGSLRLSCAASGVTFNYYGMSWIRQAPGKGLEWVASITNSGGRIYYPDSVKGRFTISRENTQKTLYLQMNSLRAEDTAVYYCTLDGRDGWVAYWGQGTLVTVSSGGGGSGGGGSGGGGSNFMLTQPSSVSGVPGQRVTISCTGNTGNIGSNYVNWYQQLPGTAPKLLIYRDDKRPSGVPDRFSGSKSGTSASLAITGFQAEDEADYYCQSYSSGFIFGGGTKLTVLGAAAGAGGDYKDDDDKGAAAHHHHHH

SEQ ID NO: 26 - protein, 8 aa, Artificial Sequence
  7000_CDR-H1
GVTFNYYG

SEQ ID NO: 27 - protein, 8 aa, Artificial Sequence
  7000_CDR-H2
ITNSGGRI

SEQ ID NO: 28 - protein, 11 aa, Artificial Sequence
  7000_CDR-H3
TLDGRDGWVAY

SEQ ID NO: 29 - protein, 8 aa, Artificial Sequence
  7000_CDR-L1
TGNIGSNY

SEQ ID NO: 30 - protein, 3 aa, Artificial Sequence
  7000_CDR-L2
RDD

SEQ ID NO: 31 - protein, 8 aa, Artificial Sequence
  7000_CDR-L3
QSYSSGFI

SEQ ID NO: 32 - DNA, 864 bp, Artificial Sequence
  C3E-3000 ORF
atgaagcacctgtggttctttctgctgctggtggccgctcccagatgggtgctgtctcaggtgcagctgcagcagtctggcgccgaactggctagacctggcgcctccgtgaagatgagctgcaaggccagcggctacaccttcacccggtacaccatgcactgggtcaagcagaggcctggacagggcctggaatggatcggctacatcaaccccagccggggctacaccaactacaaccagaagttcaaggacaaggccaccctgaccaccgacaagagcagcagcaccgcctacatgcagctgtccagcctgaccagcgaggacagcgccgtgtactactgcgcccggtactacgacgaccactactgcctggactactggggccagggcaccacactgaccgtgtctagtggtggaggcggttcaggcggaggtggcagcggcggtggcgggagtcagatcgtgctgacacagagccccgccatcatgtctgccagccctggcgagaaagtgaccatgacctgtagcgccagcagcagcgtgtcctacatgaactggtatcagcagaagtccggcaccagccccaagcggtggatctacgacacaagcaagctggcctctggcgtgcccgcccactttagaggctctggcagcggcacaagctacagcctgaccatcagcggcatggaagccgaggatgccgccacctactactgccagcagtggtccagcaaccccttcacctttggctccggcacaaagctggaaatcaagcggggcgcgtctgcggccgcaggtagcggtggtgattacaaagatgatgacgataaaggtgcagcggcgcatcaccatcatcaccac

SEQ ID NO: 33 - protein, 269 aa, Artificial Sequence
  C3E-3000 AA
QVQLQQSGAELARPGASVKMSCKASGYTFTRYTMHWVKQRPGQGLEWIGYINPSRGYTNYNQKFKDKATLTTDKSSSTAYMQLSSLTSEDSAVYYCARYYDDHYCLDYWGQGTTLTVSSGGGGSGGGGSGGGGSQIVLTQSPAIMSASPGEKVTMTCSASSSVSYMNWYQQKSGTSPKRWIYDTSKLASGVPAHFRGSGSGTSYSLTISGMEAEDAATYYCQQWSSNPFTFGSGTKLEIKRGASAAAGSGGDYKDDDDKGAAAHHHHHH

SEQ ID NO: 34 - DNA, 864 bp, Artificial Sequence
  C3E-3007 ORF
atgaagcacctgtggttctttctgctgctggtggccgctcccagatgggtgctgtctcaggtgcagctggtgcagtctggcgccgagagcaaaaagcctggcgcctccgtgaaggtgtcctgcaaggccagcggctacacctttacccggtacaccatgcactgggtgcgccaggcacctggacagggcctggaatggatgggctacatcaaccccagccggggctacaccaactacaaccagaaattcaaggaccgcgtgaccatcaccgccgacaagagcaccagcaccgcctacatggaactgagcagcctgcggagcgaggacaccgccgtgtactactgtgcccggtactacgacgaccactactgcctggactactggggccagggcacactcgtgaccgtgtctagtggtggaggcggttcaggcggaggtggcagcggcggtggcgggagtcagatccagatgacccagagccctagcagcctggccgtgtctctgggagagagagccaccatcacctgtagcgccagcagcagcgtgtcctacatgaactggtatcagcagaagcccggcaaggcccccaagcggtggatctacgataccagcaagctggcctccggcgtgcccgatagattttctggcagcggctccggcaccgacttcaccctgacaatcagctccctgcaggccgaggacgtggccacctactactgtcagcagtggtccagcaaccccttcaccttcggccagggcaccaaggtggaaatcaagcggggcgcgtctgcggccgcaggtagcggtggtgattacaaagatgatgacgataaaggtgcagcggcgcatcaccatcatcaccac

SEQ ID NO: 35 - protein, 269 aa, Artificial Sequence
  C3E-3007 AA
QVQLVQSGAESKKPGASVKVSCKASGYTFTRYTMHWVRQAPGQGLEWMGYINPSRGYTNYNQKFKDRVTITADKSTSTAYMELSSLRSEDTAVYYCARYYDDHYCLDYWGQGTLVTVSSGGGGSGGGGSGGGGSQIQMTQSPSSLAVSLGERATITCSASSSVSYMNWYQQKPGKAPKRWIYDTSKLASGVPDRFSGSGSGTDFTLTISSLQAEDVATYYCQQWSSNPFTFGQGTKVEIKRGASAAAGSGGDYKDDDDKGAAAHHHHHH

SEQ ID NO: 36 - protein, 119 aa, Artificial Sequence [sequence omitted]

SEQ ID NO: 37 - protein, 106 aa, Artificial Sequence [sequence omitted]

SEQ ID NO: 38 - protein, 119 aa, Artificial Sequence
  C3E-3007_VH AA
QVQLVQSGAESKKPGASVKVSCKASGYTFTRYTMHWVRQAPGQGLEWMGYINPSRGYTNYNQKFKDRVTITADKSTSTAYMELSSLRSEDTAVYYCARYYDDHYCLDYWGQGTLVTVSS

SEQ ID NO: 39 - protein, 106 aa, Artificial Sequence
  C3E-3007_VL AA
QIQMTQSPSSLAVSLGERATITCSASSSVSYMNWYQQKPGKAPKRWIYDTSKLASGVPDRFSGSGSGTDFTLTISSLQAEDVATYYCQQWSSNPFTFGQGTKVEIK

SEQ ID NO: 40 - DNA, 822 bp, Artificial Sequence
  HT1-11 scFv ORF
atgaagcacctgtggttctttctgctgctggtggccgctcccagatgggtgctgtctcaggtgcagctggtgcagtctggcgccgaagtgaagaaaccaggcgccagcgtgaaggtgtcctgcaaggccagcggctacacctttaccaccgccggcatgcagtgggtgcgccaggctcctggacagggcctggaatggatgggctggatcaacacccacagcggcgtgcccaaatacgccgaggacttcaagggcagagtgaccatcagcgccgacaccagcacctccacagcctacctgcagctgagcagcctgaagtccgaggacaccgccgtgtactactgcgccagaagcggcttcggcagcagctactggtacttcgacgtgtggggccagggcaccctcgtgacagtgtctagcggaggcggaggatctggcggcggaggaagtggcggagggggatccgatatccagatgacccagagccccagcagcctgtctgccagcgtgggcgacagagtgacaattacatgcaaggcctcccaggacgtgtccacagccgtggcctggtatcagcagaagcctggcaaggcccccaagctgctgatctacagcgccagctaccggtacaccggcgtgccaagcagattttccggcagcggctccggcaccgacttcaccctgacaatcagctccctgcagcccgaggatttcgccgtgtattattgccagcagcactacatcacccccctgaccttcggccaggggaccaagctggaaatcaagagaacaggcgccgctgcccaccaccaccatcaccat

SEQ ID NO: 41 - protein, 255 aa, Artificial Sequence
  HT1-11 scFv AA
QVQLVQSGAEVKKPGASVKVSCKASGYTFTTAGMQWVRQAPGQGLEWMGWINTHSGVPKYAEDFKGRVTISADTSTSTAYLQLSSLKSEDTAVYYCARSGFGSSYWYFDVWGQGTLVTVSSGGGGSGGGGSGGGGSDIQMTQSPSSLSASVGDRVTITCKASQDVSTAVAWYQQKPGKAPKLLIYSASYRYTGVPSRFSGSGSGTDFTLTISSLQPEDFAVYYCQQHYITPLTFGQGTKLEIKRTGAAAHHHHHH

SEQ ID NO: 42 - DNA, 1614 bp, Artificial Sequence
  T2C-0001 ORF
atgaaacacctgtggttcttcctcctgctggtggcagctcccagatgggtgctgagcggacaggtgcagctggtgcagtctggcgccgaagtgaagaaaccaggcgccagcgtgaaggtgtcctgcaaggccagcggctacacctttaccaccgccggcatgcagtgggtgcgccaggctcctggacagggcctggaatggatgggctggatcaacacccacagcggcgtgcccaaatacgccgaggacttcaagggcagagtgaccatcagcgccgacaccagcacctccacagcctacctgcagctgagcagcctgaagtccgaggacaccgccgtgtactactgcgccagaagcggcttcggcagcagctactggtacttcgacgtgtggggccagggcaccctcgtgacagtgtctagcggaggcggaggatctggcggcggaggaagtggcggagggggatccgatatccagatgacccagagccccagcagcctgtctgccagcgtgggcgacagagtgacaattacatgcaaggcctcccaggacgtgtccacagccgtggcctggtatcagcagaagcctggcaaggcccccaagctgctgatctacagcgccagctaccggtacaccggcgtgccaagcagattttccggcagcggctccggcaccgacttcaccctgacaatcagctccctgcagcccgaggatttcgccgtgtattattgccagcagcactacatcacccccctgaccttcggccaggggaccaagctggaaatcaagagaacagggggaggcggttcagaagtgcagctggtggaatccggggggggcctggtgcagcctggggggagcctgagactgagttgtgccgcctctggggtgacatttaactactatggcatgtcttggatccgccaggcacctggaaagggcctggagtgggtggccagcatcactaattccggcgggcgaatctactatcccgacagcgtcaagggcaggttcacaatttcccgcgagaacacacagaaaactctgtacctgcagatgaatagcctgagagccgaagatacagctgtgtactattgcactctggacggcagggatgggtgggtcgcctattgggggcagggaaccctggtgacagtcagctccggaggaggaggatctggcggaggaggcagtgggggaggcgggtcaaactttatgctgacccagccccacagtgtgtcagagagccctggcaagactgtcaccatctcttgtaaaaggaacaccggaaatattggcagtaactacgtgaattggtatcagcagcatgaagggtctagtccaaccacaatcatctaccgggacgataagagacccgacggggtgtccgatcgattctccggatctatcgaccggtcaagcaagagtgcttcactgaccattagcaatctgaaaacagaggacgaagcagattacttttgccagtcctattcctctggcttcatctttggaggcgggactaaactgaccgtgctgggcgcggccgcaggtgcaggtggtgattacaaagatgatgacgataaaggtgcagcggcgcatcaccatcatcaccac

SEQ ID NO: 43 - protein, 519 aa, Artificial Sequence
  T2C-0001 AA
GQVQLVQSGAEVKKPGASVKVSCKASGYTFTTAGMQWVRQAPGQGLEWMGWINTHSGVPKYAEDFKGRVTISADTSTSTAYLQLSSLKSEDTAVYYCARSGFGSSYWYFDVWGQGTLVTVSSGGGGSGGGGSGGGGSDIQMTQSPSSLSASVGDRVTITCKASQDVSTAVAWYQQKPGKAPKLLIYSASYRYTGVPSRFSGSGSGTDFTLTISSLQPEDFAVYYCQQHYITPLTFGQGTKLEIKRTGGGGSEVQLVESGGGLVQPGGSLRLSCAASGVTFNYYGMSWIRQAPGKGLEWVASITNSGGRIYYPDSVKGRFTISRENTQKTLYLQMNSLRAEDTAVYYCTLDGRDGWVAYWGQGTLVTVSSGGGGSGGGGSGGGGSNFMLTQPHSVSESPGKTVTISCKRNTGNIGSNYVNWYQQHEGSSPTTIIYRDDKRPDGVSDRFSGSIDRSSKSASLTISNLKTEDEADYFCQSYSSGFIFGGGTKLTVLGAAAGAGGDYKDDDDKGAAAHHHHHH

SEQ ID NO: 44 - DNA, 1647 bp, Artificial Sequence
  T2C-0003 ORF
atgaaacacctgtggttcttcctcctgctggtggcagctcccagatgggtgctgagcggacaggtgcagctggtgcagtctggcgccgaagtgaagaaaccaggcgccagcgtgaaggtgtcctgcaaggccagcggctacacctttaccaccgccggcatgcagtgggtgcgccaggctcctggacagggcctggaatggatgggctggatcaacacccacagcggcgtgcccaaatacgccgaggacttcaagggcagagtgaccatcagcgccgacaccagcacctccacagcctacctgcagctgagcagcctgaagtccgaggacaccgccgtgtactactgcgccagaagcggcttcggcagcagctactggtacttcgacgtgtggggccagggcaccctcgtgacagtgtctagcggaggcggaggatctggcggcggaggaagtggcggagggggatccgatatccagatgacccagagccccagcagcctgtctgccagcgtgggcgacagagtgacaattacatgcaaggcctcccaggacgtgtccacagccgtggcctggtatcagcagaagcctggcaaggcccccaagctgctgatctacagcgccagctaccggtacaccggcgtgccaagcagattttccggcagcggctccggcaccgacttcaccctgacaatcagctccctgcagcccgaggatttcgccgtgtattattgccagcagcactacatcacccccctgaccttcggccaggggaccaagctggaaatcaagagaacagggggaggcggttcagaagtgcagctggtggaatccggcggaggcctggtccagcctggcggcagcctgaaactgagctgcgccgccagcggcttcaccttcaacaaatacgccatgaactgggtccgccaggctcctggaaagggactcgagtgggtggcccggatcagaagcaagtacaacaactacgccacctactacgccgacagcgtgaaggaccggttcaccatcagccgggacgacagcaagaacaccgcctacctgcagatgaacaacctgaaaaccgaggacacagccgtgtactactgcgtgcggcacggcaacttcggcaacagctacatcagctactgggcctattggggacagggaacactcgtgacagtgtccagtggcggaggcggcagtggtgggggaggaagcggaggtggcggatctcagaccgtggtcacccaggaacccagcctgacagtcagccctggaggcaccgtgaccctgacctgtggaagcagcacaggcgccgtgaccagcggctactaccccaactgggtgcagcagaagcccggccaggctcctagaggcctgatcggcggcaccaagtttctggcccctggcacccctgcccggttctctggatctctgctgggcggcaaggccgccctgacactgagcggagtgcagcccgaggacgaggccgagtactactgtgccctgtggtacagcaacagatgggtgttcggcggagggaccaagctgaccgtgctgggcagcggcgcgtctgcggccgcaggtagcggtggtgattacaaagatgatgacgataaaggtgcagcggcgcatcaccatcatcaccac

SEQ ID NO: 45 - protein, 530 aa, Artificial Sequence
  T2C-0003 AA
GQVQLVQSGAEVKKPGASVKVSCKASGYTFTTAGMQWVRQAPGQGLEWMGWINTHSGVPKYAEDFKGRVTISADTSTSTAYLQLSSLKSEDTAVYYCARSGFGSSYWYFDVWGQGTLVTVSSGGGGSGGGGSGGGGSDIQMTQSPSSLSASVGDRVTITCKASQDVSTAVAWYQQKPGKAPKLLIYSASYRYTGVPSRFSGSGSGTDFTLTISSLQPEDFAVYYCQQHYITPLTFGQGTKLEIKRTGGGGSEVQLVESGGGLVQPGGSLKLSCAASGFTFNKYAMNWVRQAPGKGLEWVARIRSKYNNYATYYADSVKDRFTISRDDSKNTAYLQMNNLKTEDTAVYYCVRHGNFGNSYISYWAYWGQGTLVTVSSGGGGSGGGGSGGGGSQTVVTQEPSLTVSPGGTVTLTCGSSTGAVTSGYYPNWVQQKPGQAPRGLIGGTKFLAPGTPARFSGSLLGGKAALTLSGVQPEDEAEYYCALWYSNRWVFGGGTKLTVLGSGASAAAGSGGDYKDDDDKGAAAHHHHHH

SEQ ID NO: 46 - DNA, 1614 bp, Artificial Sequence
  T2C-0005 ORF
atgaagcacctgtggttcttcctcctgctggtggcagctcccagatgggtgctgagcggacaggtgcagctggtgcagtctggcgccgaagtgaagaaaccaggcgccagcgtgaaggtgtcctgcaaggccagcggctacacctttaccaccgccggcatgcagtgggtgcgccaggctcctggacagggcctggaatggatgggctggatcaacacccacagcggcgtgcccaaatacgccgaggacttcaagggcagagtgaccatcagcgccgacaccagcacctccacagcctacctgcagctgagcagcctgaagtccgaggacaccgccgtgtactactgcgccagaagcggcttcggcagcagctactggtacttcgacgtgtggggccagggcaccctcgtgacagtgtctagcggaggcggaggatctggcggcggaggaagtggcggagggggatccgatatccagatgacccagagccccagcagcctgtctgccagcgtgggcgacagagtgacaattacatgcaaggcctcccaggacgtgtccacagccgtggcctggtatcagcagaagcctggcaaggcccccaagctgctgatctacagcgccagctaccggtacaccggcgtgccaagcagattttccggcagcggctccggcaccgacttcaccctgacaatcagctccctgcagcccgaggatttcgccgtgtattattgccagcagcactacatcacccccctgaccttcggccaggggaccaagctggaaatcaagagaacagggggaggcggttcagaagtgcagctggtggaatccggggggggcctggtgcagcctggggggagcctgagactgagttgtgccgcctctggggtgacatttaactactatggcatgtcttggatccgccaggcacctggaaagggcctggagtgggtggccagcatcactaattccggcgggcgaatctactatcccgacagcgtcaagggcaggttcacaatttcccgcgagaacacacagaaaactctgtacctgcagatgaatagcctgagagccgaagatacagctgtgtactattgcactctggacggcagggatgggtgggtcgcctattgggggcagggaaccctggtgacagtcagctccggaggaggaggatctggcggaggaggcagtgggggaggcgggtcaatggcccaggctgtgctcactcagccgtcctctgtttctggcgtacctggccaacgggtgaccattagctgtaaaaggaataccgggaatatcgggtctaactacgtgaactggtatcagcagcttccagggacagctcccaagttgctgatctatcgcgacgacaaaagaccctcaggggtccctgaccgatttagtggcagcaaaagcggtacttccgcttccctggcgataaccggctttcaggccgaagatgaggcagactactattgccagtcatattccagcggcttcatcttcggaggcggaactaagctgacagtgttgggcgcggccgcaggtgcaggtggtgattacaaagatgatgacgataaaggtgcagcggcgcatcaccatcatcaccac

SEQ ID NO: 47 - protein, 519 aa, Artificial Sequence
  T2C-0005 AA
GQVQLVQSGAEVKKPGASVKVSCKASGYTFTTAGMQWVRQAPGQGLEWMGWINTHSGVPKYAEDFKGRVTISADTSTSTAYLQLSSLKSEDTAVYYCARSGFGSSYWYFDVWGQGTLVTVSSGGGGSGGGGSGGGGSDIQMTQSPSSLSASVGDRVTITCKASQDVSTAVAWYQQKPGKAPKLLIYSASYRYTGVPSRFSGSGSGTDFTLTISSLQPEDFAVYYCQQHYITPLTFGQGTKLEIKRTGGGGSEVQLVESGGGLVQPGGSLRLSCAASGVTFNYYGMSWIRQAPGKGLEWVASITNSGGRIYYPDSVKGRFTISRENTQKTLYLQMNSLRAEDTAVYYCTLDGRDGWVAYWGQGTLVTVSSGGGGSGGGGSGGGGSMAQAVLTQPSSVSGVPGQRVTISCKRNTGNIGSNYVNWYQQLPGTAPKLLIYRDDKRPSGVPDRFSGSKSGTSASLAITGFQAEDEADYYCQSYSSGFIFGGGTKLTVLGAAAGAGGDYKDDDDKGAAAHHHHHH

SEQ ID NO: 48 - DNA, 1608 bp, Artificial Sequence
  T2C-0006 ORF
atgaagcacctgtggttcttcctcctgctggtggcagctcccagatgggtgctgagcggacaggtgcagctggtgcagtctggcgccgaagtgaagaaaccaggcgccagcgtgaaggtgtcctgcaaggccagcggctacacctttaccaccgccggcatgcagtgggtgcgccaggctcctggacagggcctggaatggatgggctggatcaacacccacagcggcgtgcccaaatacgccgaggacttcaagggcagagtgaccatcagcgccgacaccagcacctccacagcctacctgcagctgagcagcctgaagtccgaggacaccgccgtgtactactgcgccagaagcggcttcggcagcagctactggtacttcgacgtgtggggccagggcaccctcgtgacagtgtctagcggaggcggaggatctggcggcggaggaagtggcggagggggatccgatatccagatgacccagagccccagcagcctgtctgccagcgtgggcgacagagtgacaattacatgcaaggcctcccaggacgtgtccacagccgtggcctggtatcagcagaagcctggcaaggcccccaagctgctgatctacagcgccagctaccggtacaccggcgtgccaagcagattttccggcagcggctccggcaccgacttcaccctgacaatcagctccctgcagcccgaggatttcgccgtgtattattgccagcagcactacatcacccccctgaccttcggccaggggaccaagctggaaatcaagagaacagggggaggcggttcagaagtgcagctggtggaatccggggggggcctggtgcagcctggggggagcctgagactgagttgtgccgcctctggggtgacatttaactactatggcatgtcttggatccgccaggcacctggaaagggcctggagtgggtggccagcatcactaattccggcgggcgaatctactatcccgacagcgtcaagggcaggttcacaatttcccgcgagaacacacagaaaactctgtacctgcagatgaatagcctgagagccgaagatacagctgtgtactattgcactctggacggcagggatgggtgggtcgcctattgggggcagggaaccctggtgacagtcagctccggaggaggaggatctggcggaggaggcagtgggggaggcgggtcaaactttatgctcactcagccgtcctctgtttctggcgtacctggccaacgggtgaccattagctgtacgggtaataccgggaatatcgggtctaactacgtgaactggtatcagcagcttccagggacagctcccaagttgctgatctatcgcgacgacaaaagaccctcaggggtccctgaccgatttagtggcagcaaaagcggtacttccgcttccctggcgataaccggctttcaggccgaagatgaggcagactactattgccagtcatattccagcggcttcatcttcggaggcggaactaagctgacagtgttgggcgcggccgcaggtgcaggtggtgattacaaagatgatgacgataaaggtgcagcggcgcatcaccatcatcaccac

SEQ ID NO: 49 - protein, 517 aa, Artificial Sequence
  T2C-0006 AA
GQVQLVQSGAEVKKPGASVKVSCKASGYTFTTAGMQWVRQAPGQGLEWMGWINTHSGVPKYAEDFKGRVTISADTSTSTAYLQLSSLKSEDTAVYYCARSGFGSSYWYFDVWGQGTLVTVSSGGGGSGGGGSGGGGSDIQMTQSPSSLSASVGDRVTITCKASQDVSTAVAWYQQKPGKAPKLLIYSASYRYTGVPSRFSGSGSGTDFTLTISSLQPEDFAVYYCQQHYITPLTFGQGTKLEIKRTGGGGSEVQLVESGGGLVQPGGSLRLSCAASGVTFNYYGMSWIRQAPGKGLEWVASITNSGGRIYYPDSVKGRFTISRENTQKTLYLQMNSLRAEDTAVYYCTLDGRDGWVAYWGQGTLVTVSSGGGGSGGGGSGGGGSNFMLTQPSSVSGVPGQRVTISCTGNTGNIGSNYVNWYQQLPGTAPKLLIYRDDKRPSGVPDRFSGSKSGTSASLAITGFQAEDEADYYCQSYSSGFIFGGGTKLTVLGAAAGAGGDYKDDDDKGAAAHHHHHH

SEQ ID NO: 50 - DNA, 37 bp, Artificial Sequence
  Nhe-polyC-S
  misc_feature (37)..(37): n is a, c, g or t
gctagcgctaccggactcagatcccccccccccccdn

SEQ ID NO: 51 - DNA, 28 bp, Artificial Sequence
  rIg gamma-AS1
tcactgagctggtgagagtgtagagccc

SEQ ID NO: 52 - DNA, 28 bp, Artificial Sequence
  rIg gamma-AS2
tcaccgagctgctgagggtgtagagccc

SEQ ID NO: 53 - DNA, 37 bp, Artificial Sequence; identical to SEQ ID NO: 50
  Nhe-polyC-S2
  misc_feature (37)..(37): n is a, c, g or t

SEQ ID NO: 54 - DNA, 26 bp, Artificial Sequence
  rIgL-AS1
ttccacatcactcgggtagaaatcag

SEQ ID NO: 55 - DNA, 28 bp, Artificial Sequence
  rIgL-AS2
taacaccagggtagaaatctgtcaccat

SEQ ID NO: 56 - DNA, 19 bp, Artificial Sequence
  rIg gamma-seq
ctggctcagggaaatagcc

SEQ ID NO: 57 - DNA, 18 bp, Artificial Sequence
  rIgL-seq1
tccctggagctcctcagt

SEQ ID NO: 58 - DNA, 18 bp, Artificial Sequence
  rIgL-seq2
gccttgtcagtcttgagc

SEQ ID NO: 59 - DNA, 864 bp, Artificial Sequence
  C3E-7078 ORF
atgaaacacctgtggttcttcctcctgctggtggcagctcccagatgggtgctgagcggagaagtgcagctggtggaatccggggggggcctggtgcagcctggggggagcctgagactgagttgtgccgcctctggggtgacatttaactactatggcatgtcttggatccgccaggcacctggaaagggcctggagtgggtggccagcatcactaggtccggcgggcgaatctactatcccgacagcgtcaagggcaggttcacaatttcccgcgagaacacacagaaaactctgtacctgcagatgaatagcctgagagccgaagatacagctgtgtactattgcactctggacggcagggatgggtgggtcgcctattgggggcagggaaccctggtgacagtcagctccggaggaggaggatctggcggaggaggcagtgggggaggcgggtcaaactttatgctgacccagccccacagtgtgtcagagagccctggcaagactgtcaccatctcttgtaaaaggaacaccggaaatattggcagtaactacgtgaattggtatcagcagcatgaagggtctagtccaaccacaatcatctaccgggacgataagagacccgacggggtgtccgatcgattctccggatctatcgaccggtcaagcaagagtgcttcactgaccattagcaatctgaaaacagaggacgaagcagattacttttgccagtcctattcctctggcttcatctttggaggcgggactaaactgaccgtgctgggcgcggccgcaggtgcaggtggtgattacaaagatgatgacgataaaggtgcagcggcgcatcaccatcatcaccac

SEQ ID NO: 60 - protein, 269 aa, Artificial Sequence
  C3E-7078 AA
GEVQLVESGGGLVQPGGSLRLSCAASGVTFNYYGMSWIRQAPGKGLEWVASITRSGGRIYYPDSVKGRFTISRENTQKTLYLQMNSLRAEDTAVYYCTLDGRDGWVAYWGQGTLVTVSSGGGGSGGGGSGGGGSNFMLTQPHSVSESPGKTVTISCKRNTGNIGSNYVNWYQQHEGSSPTTIIYRDDKRPDGVSDRFSGSIDRSSKSASLTISNLKTEDEADYFCQSYSSGFIFGGGTKLTVLGAAAGAGGDYKDDDDKGAAAHHHHHH

SEQ ID NO: 61 - DNA, 864 bp, Artificial Sequence
  C3E-7079 ORF
atgaaacacctgtggttcttcctcctgctggtggcagctcccagatgggtgctgagcggagaagtgcagctggtggaatccggggggggcctggtgcagcctggggggagcctgagactgagttgtgccgcctctggggtgacatttaactactatggcatgtcttggatccgccaggcacctggaaagggcctggagtgggtggccagcatcacttcttccggcgggcgaatctactatcccgacagcgtcaagggcaggttcacaatttcccgcgagaacacacagaaaactctgtacctgcagatgaatagcctgagagccgaagatacagctgtgtactattgcactctggacggcagggatgggtgggtcgcctattgggggcagggaaccctggtgacagtcagctccggaggaggaggatctggcggaggaggcagtgggggaggcgggtcaaactttatgctgacccagccccacagtgtgtcagagagccctggcaagactgtcaccatctcttgtaaaaggaacaccggaaatattggcagtaactacgtgaattggtatcagcagcatgaagggtctagtccaaccacaatcatctaccgggacgataagagacccgacggggtgtccgatcgattctccggatctatcgaccggtcaagcaagagtgcttcactgaccattagcaatctgaaaacagaggacgaagcagattacttttgccagtcctattcctctggcttcatctttggaggcgggactaaactgaccgtgctgggcgcggccgcaggtgcaggtggtgattacaaagatgatgacgataaaggtgcagcggcgcatcaccatcatcaccac

SEQ ID NO: 62 - protein, 269 aa, Artificial Sequence
  C3E-7079 AA
GEVQLVESGGGLVQPGGSLRLSCAASGVTFNYYGMSWIRQAPGKGLEWVASITSSGGRIYYPDSVKGRFTISRENTQKTLYLQMNSLRAEDTAVYYCTLDGRDGWVAYWGQGTLVTVSSGGGGSGGGGSGGGGSNFMLTQPHSVSESPGKTVTISCKRNTGNIGSNYVNWYQQHEGSSPTTIIYRDDKRPDGVSDRFSGSIDRSSKSASLTISNLKTEDEADYFCQSYSSGFIFGGGTKLTVLGAAAGAGGDYKDDDDKGAAAHHHHHH

SEQ ID NO: 63 - DNA, 858 bp, Artificial Sequence
  C3E-7085 ORF
atgaaacacctgtggttcttcctcctgctggtggcagctcccagatgggtgctgagcggagaagtgcagctggtggaatccggggggggcctggtgcagcctggggggagcctgagactgagttgtgccgcctctggggtgacatttaactactatggcatgtcttggatccgccaggcacctggaaagggcctggagtgggtggccagcatcactaggtccggcgggcgaatctactatcccgacagcgtcaagggcaggttcacaatttcccgcgagaacacacagaaaactctgtacctgcagatgaatagcctgagagccgaagatacagctgtgtactattgcactctggacggcagggatgggtgggtcgcctattgggggcagggaaccctggtgacagtcagctccggaggaggaggatctggcggaggaggcagtgggggaggcgggtcaaactttatgctcactcagccgtcctctgtttctggcgtacctggccaacgggtgaccattagctgtacgggtaataccgggaatatcgggtctaactacgtgaactggtatcagcagcttccagggacagctcccaagttgctgatctatcgcgacgacaaaagaccctcaggggtccctgaccgatttagtggcagcaaaagcggtacttccgcttccctggcgataaccggctttcaggccgaagatgaggcagactactattgccagtcatattccagcggcttcatcttcggaggcggaactaagctgacagtgttgggcgcggccgcaggtgcaggtggtgattacaaagatgatgacgataaaggtgcagcggcgcatcaccatcatcaccac

SEQ ID NO: 64 - protein, 267 aa, Artificial Sequence
  C3E-7085 AA
GEVQLVESGGGLVQPGGSLRLSCAASGVTFNYYGMSWIRQAPGKGLEWVASITRSGGRIYYPDSVKGRFTISRENTQKTLYLQMNSLRAEDTAVYYCTLDGRDGWVAYWGQGTLVTVSSGGGGSGGGGSGGGGSNFMLTQPSSVSGVPGQRVTISCTGNTGNIGSNYVNWYQQLPGTAPKLLIYRDDKRPSGVPDRFSGSKSGTSASLAITGFQAEDEADYYCQSYSSGFIFGGGTKLTVLGAAAGAGGDYKDDDDKGAAAHHHHHH

SEQ ID NO: 65 - DNA, 864 bp, Artificial Sequence
  C3E-7086 ORF
atgaaacacctgtggttcttcctcctgctggtggcagctcccagatgggtgctgagcggagaagtgcagctggtggaatccggggggggcctggtgcagcctggggggagcctgagactgagttgtgccgcctctggggtgacatttaactactatggcatgtcttggatccgccaggcacctggaaagggcctggagtgggtggccagcatcactaggtccggcgggcgaatctactatcccgacagcgtcaagggcaggttcacaatttcccgcgagaacacacagaaaactctgtacctgcagatgaatagcctgagagccgaagatacagctgtgtactattgcactctggacggcagggatgggtgggtcgcctattgggggcagggaaccctggtgacagtcagctccggaggaggaggatctggcggaggaggcagtgggggaggcgggtcaaactttatgctgacccagccccacagtgtgtcagagagccctggcaagactgtcaccatctcttgtaaaaggaacaccggaaatattggcagtaactacgtgaattggtatcagcagcatgaagggtctagtccaaccacaatcatctaccggggcgataagagacccgacggggtgtccgatcgattctccggatctatcgaccggtcaagcaagagtgcttcactgaccattagcaatctgaaaacagaggacgaagcagattacttttgccagtcctattcctctggcttcatctttggaggcgggactaaactgaccgtgctgggcgcggccgcaggtgcaggtggtgattacaaagatgatgacgataaaggtgcagcggcgcatcaccatcatcaccac

SEQ ID NO: 66 - protein, 269 aa, Artificial Sequence
  C3E-7086 AA
GEVQLVESGGGLVQPGGSLRLSCAASGVTFNYYGMSWIRQAPGKGLEWVASITRSGGRIYYPDSVKGRFTISRENTQKTLYLQMNSLRAEDTAVYYCTLDGRDGWVAYWGQGTLVTVSSGGGGSGGGGSGGGGSNFMLTQPHSVSESPGKTVTISCKRNTGNIGSNYVNWYQQHEGSSPTTIIYRGDKRPDGVSDRFSGSIDRSSKSASLTISNLKTEDEADYFCQSYSSGFIFGGGTKLTVLGAAAGAGGDYKDDDDKGAAAHHHHHH

SEQ ID NO: 67 - DNA, 864 bp, Artificial Sequence
  C3E-7087 ORF
atgaaacacctgtggttcttcctcctgctggtggcagctcccagatgggtgctgagcggagaagtgcagctggtggaatccggggggggcctggtgcagcctggggggagcctgagactgagttgtgccgcctctggggtgacatttaactactatggcatgtcttggatccgccaggcacctggaaagggcctggagtgggtggccagcatcactaggtccggcgggcgaatctactatcccgacagcgtcaagggcaggttcacaatttcccgcgagaacacacagaaaactctgtacctgcagatgaatagcctgagagccgaagatacagctgtgtactattgcactctggacggcagggatgggtgggtcgcctattgggggcagggaaccctggtgacagtcagctccggaggaggaggatctggcggaggaggcagtgggggaggcgggtcaaactttatgctgacccagccccacagtgtgtcagagagccctggcaagactgtcaccatctcttgtaaaaggaacaccggaaatattggcagtaactacgtgaattggtatcagcagcatgaagggtctagtccaaccacaatcatctaccggcaggataagagacccgacggggtgtccgatcgattctccggatctatcgaccggtcaagcaagagtgcttcactgaccattagcaatctgaaaacagaggacgaagcagattacttttgccagtcctattcctctggcttcatctttggaggcgggactaaactgaccgtgctgggcgcggccgcaggtgcaggtggtgattacaaagatgatgacgataaaggtgcagcggcgcatcaccatcatcaccac

SEQ ID NO: 68 - protein, 269 aa, Artificial Sequence
  C3E-7087 AA
GEVQLVESGGGLVQPGGSLRLSCAASGVTFNYYGMSWIRQAPGKGLEWVASITRSGGRIYYPDSVKGRFTISRENTQKTLYLQMNSLRAEDTAVYYCTLDGRDGWVAYWGQGTLVTVSSGGGGSGGGGSGGGGSNFMLTQPHSVSESPGKTVTISCKRNTGNIGSNYVNWYQQHEGSSPTTIIYRQDKRPDGVSDRFSGSIDRSSKSASLTISNLKTEDEADYFCQSYSSGFIFGGGTKLTVLGAAAGAGGDYKDDDDKGAAAHHHHHH

SEQ ID NO: 69 - DNA, 864 bp, Artificial Sequence
  C3E-7088 ORF
atgaaacacctgtggttcttcctcctgctggtggcagctcccagatgggtgctgagcggagaagtgcagctggtggaatccggggggggcctggtgcagcctggggggagcctgagactgagttgtgccgcctctggggtgacatttaactactatggcatgtcttggatccgccaggcacctggaaagggcctggagtgggtggccagcatcactaggtccggcgggcgaatctactatcccgacagcgtcaagggcaggttcacaatttcccgcgagaacacacagaaaactctgtacctgcagatgaatagcctgagagccgaagatacagctgtgtactattgcactctggacggcagggatgggtgggtcgcctattgggggcagggaaccctggtgacagtcagctccggaggaggaggatctggcggaggaggcagtgggggaggcgggtcaaactttatgctgacccagccccacagtgtgtcagagagccctggcaagactgtcaccatctcttgtaaaaggaacaccggaaatattggcagtaactacgtgaattggtatcagcagcatgaagggtctagtccaaccacaatcatctaccggaacgataagagacccgacggggtgtccgatcgattctccggatctatcgaccggtcaagcaagagtgcttcactgaccattagcaatctgaaaacagaggacgaagcagattacttttgccagtcctattcctctggcttcatctttggaggcgggactaaactgaccgtgctgggcgcggccgcaggtgcaggtggtgattacaaagatgatgacgataaaggtgcagcggcgcatcaccatcatcaccac

SEQ ID NO: 70 - protein, 269 aa, Artificial Sequence
  C3E-7088 AA
GEVQLVESGGGLVQPGGSLRLSCAASGVTFNYYGMSWIRQAPGKGLEWVASITRSGGRIYYPDSVKGRFTISRENTQKTLYLQMNSLRAEDTAVYYCTLDGRDGWVAYWGQGTLVTVSSGGGGSGGGGSGGGGSNFMLTQPHSVSESPGKTVTISCKRNTGNIGSNYVNWYQQHEGSSPTTIIYRNDKRPDGVSDRFSGSIDRSSKSASLTISNLKTEDEADYFCQSYSSGFIFGGGTKLTVLGAAAGAGGDYKDDDDKGAAAHHHHHH

SEQ ID NO: 71 - DNA, 864 bp, Artificial Sequence
  C3E-7089 ORF
atgaaacacctgtggttcttcctcctgctggtggcagctcccagatgggtgctgagcggagaagtgcagctggtggaatccggggggggcctggtgcagcctggggggagcctgagactgagttgtgccgcctctggggtgacatttaactactatggcatgtcttggatccgccaggcacctggaaagggcctggagtgggtggccagcatcactaggtccggcgggcgaatctactatcccgacagcgtcaagggcaggttcacaatttcccgcgagaacacacagaaaactctgtacctgcagatgaatagcctgagagccgaagatacagctgtgtactattgcactctggacggcagggatgggtgggtcgcctattgggggcagggaaccctggtgacagtcagctccggaggaggaggatctggcggaggaggcagtgggggaggcgggtcaaactttatgctgacccagccccacagtgtgtcagagagccctggcaagactgtcaccatctcttgtaaaaggaacaccggaaatattggcagtaactacgtgaattggtatcagcagcatgaagggtctagtccaaccacaatcatctaccggagcgataagagacccgacggggtgtccgatcgattctccggatctatcgaccggtcaagcaagagtgcttcactgaccattagcaatctgaaaacagaggacgaagcagattacttttgccagtcctattcctctggcttcatctttggaggcgggactaaactgaccgtgctgggcgcggccgcaggtgcaggtggtgattacaaagatgatgacgataaaggtgcagcggcgcatcaccatcatcaccac

SEQ ID NO: 72 - protein, 269 aa, Artificial Sequence
  C3E-7089 AA
GEVQLVESGGGLVQPGGSLRLSCAASGVTFNYYGMSWIRQAPGKGLEWVASITRSGGRIYYPDSVKGRFTISRENTQKTLYLQMNSLRAEDTAVYYCTLDGRDGWVAYWGQGTLVTVSSGGGGSGGGGSGGGGSNFMLTQPHSVSESPGKTVTISCKRNTGNIGSNYVNWYQQHEGSSPTTIIYRSDKRPDGVSDRFSGSIDRSSKSASLTISNLKTEDEADYFCQSYSSGFIFGGGTKLTVLGAAAGAGGDYKDDDDKGAAAHHHHHH

SEQ ID NO: 73 - DNA, 864 bp, Artificial Sequence
  C3E-7090 ORF
atgaaacacctgtggttcttcctcctgctggtggcagctcccagatgggtgctgagcggagaagtgcagctggtggaatccggggggggcctggtgcagcctggggggagcctgagactgagttgtgccgcctctggggtgacatttaactactatggcatgtcttggatccgccaggcacctggaaagggcctggagtgggtggccagcatcactaggtccggcgggcgaatctactatcccgacagcgtcaagggcaggttcacaatttcccgcgagaacacacagaaaactctgtacctgcagatgaatagcctgagagccgaagatacagctgtgtactattgcactctggacggcagggatgggtgggtcgcctattgggggcagggaaccctggtgacagtcagctccggaggaggaggatctggcggaggaggcagtgggggaggcgggtcaaactttatgctgacccagccccacagtgtgtcagagagccctggcaagactgtcaccatctcttgtaaaaggaacaccggaaatattggcagtaactacgtgaattggtatcagcagcatgaagggtctagtccaaccacaatcatctaccgggccgataagagacccgacggggtgtccgatcgattctccggatctatcgaccggtcaagcaagagtgcttcactgaccattagcaatctgaaaacagaggacgaagcagattacttttgccagtcctattcctctggcttcatctttggaggcgggactaaactgaccgtgctgggcgcggccgcaggtgcaggtggtgattacaaagatgatgacgataaaggtgcagcggcgcatcaccatcatcaccac

SEQ ID NO: 74 - protein, 269 aa, Artificial Sequence
  C3E-7090 AA
GEVQLVESGGGLVQPGGSLRLSCAASGVTFNYYGMSWIRQAPGKGLEWVASITRSGGRIYYPDSVKGRFTISRENTQKTLYLQMNSLRAEDTAVYYCTLDGRDGWVAYWGQGTLVTVSSGGGGSGGGGSGGGGSNFMLTQPHSVSESPGKTVTISCKRNTGNIGSNYVNWYQQHEGSSPTTIIYRADKRPDGVSDRFSGSIDRSSKSASLTISNLKTEDEADYFCQSYSSGFIFGGGTKLTVLGAAAGAGGDYKDDDDKGAAAHHHHHH

SEQ ID NO: 75 - DNA, 864 bp, Artificial Sequence
  C3E-7091 ORF
atgaaacacctgtggttcttcctcctgctggtggcagctcccagatgggtgctgagcggagaagtgcagctggtggaatccggggggggcctggtgcagcctggggggagcctgagactgagttgtgccgcctctggggtgacatttaactactatggcatgtcttggatccgccaggcacctggaaagggcctggagtgggtggccagcatcacttcttccggcgggcgaatctactatcccgacagcgtcaagggcaggttcacaatttcccgcgagaacacacagaaaactctgtacctgcagatgaatagcctgagagccgaagatacagctgtgtactattgcactctggacggcagggatgggtgggtcgcctattgggggcagggaaccctggtgacagtcagctccggaggaggaggatctggcggaggaggcagtgggggaggcgggtcaaactttatgctgacccagccccacagtgtgtcagagagccctggcaagactgtcaccatctcttgtaaaaggaacaccggaaatattggcagtaactacgtgaattggtatcagcagcatgaagggtctagtccaaccacaatcatctaccggggcgataagagacccgacggggtgtccgatcgattctccggatctatcgaccggtcaagcaagagtgcttcactgaccattagcaatctgaaaacagaggacgaagcagattacttttgccagtcctattcctctggcttcatctttggaggcgggactaaactgaccgtgctgggcgcggccgcaggtgcaggtggtgattacaaagatgatgacgataaaggtgcagcggcgcatcaccatcatcaccac

SEQ ID NO: 76 - protein, 269 aa, Artificial Sequence
  C3E-7091 AA
GEVQLVESGGGLVQPGGSLRLSCAASGVTFNYYGMSWIRQAPGKGLEWVASITSSGGRIYYPDSVKGRFTISRENTQKTLYLQMNSLRAEDTAVYYCTLDGRDGWVAYWGQGTLVTVSSGGGGSGGGGSGGGGSNFMLTQPHSVSESPGKTVTISCKRNTGNIGSNYVNWYQQHEGSSPTTIIYRGDKRPDGVSDRFSGSIDRSSKSASLTISNLKTEDEADYFCQSYSSGFIFGGGTKLTVLGAAAGAGGDYKDDDDKGAAAHHHHHH

SEQ ID NO: 77 - DNA, 864 bp, Artificial Sequence
  C3E-7092 ORF
atgaaacacctgtggttcttcctcctgctggtggcagctcccagatgggtgctgagcggagaagtgcagctggtggaatccggggggggcctggtgcagcctggggggagcctgagactgagttgtgccgcctctggggtgacatttaactactatggcatgtcttggatccgccaggcacctggaaagggcctggagtgggtggccagcatcacttcttccggcgggcgaatctactatcccgacagcgtcaagggcaggttcacaatttcccgcgagaacacacagaaaactctgtacctgcagatgaatagcctgagagccgaagatacagctgtgtactattgcactctggacggcagggatgggtgggtcgcctattgggggcagggaaccctggtgacagtcagctccggaggaggaggatctggcggaggaggcagtgggggaggcgggtcaaactttatgctgacccagccccacagtgtgtcagagagccctggcaagactgtcaccatctcttgtaaaaggaacaccggaaatattggcagtaactacgtgaattggtatcagcagcatgaagggtctagtccaaccacaatcatctaccggcaggataagagacccgacggggtgtccgatcgattctccggatctatcgaccggtcaagcaagagtgcttcactgaccattagcaatctgaaaacagaggacgaagcagattacttttgccagtcctattcctctggcttcatctttggaggcgggactaaactgaccgtgctgggcgcggccgcaggtgcaggtggtgattacaaagatgatgacgataaaggtgcagcggcgcatcaccatcatcaccac

SEQ ID NO: 78 - protein, 269 aa, Artificial Sequence
  C3E-7092 AA
GEVQLVESGGGLVQPGGSLRLSCAASGVTFNYYGMSWIRQAPGKGLEWVASITSSGGRIYYPDSVKGRFTISRENTQKTLYLQMNSLRAEDTAVYYCTLDGRDGWVAYWGQGTLVTVSSGGGGSGGGGSGGGGSNFMLTQPHSVSESPGKTVTISCKRNTGNIGSNYVNWYQQHEGSSPTTIIYRQDKRPDGVSDRFSGSIDRSSKSASLTISNLKTEDEADYFCQSYSSGFIFGGGTKLTVLGAAAGAGGDYKDDDDKGAAAHHHHHH

SEQ ID NO: 79 - DNA, 864 bp, Artificial Sequence
  C3E-7093 ORF
atgaaacacctgtggttcttcctcctgctggtggcagctcccagatgggtgctgagcggagaagtgcagctggtggaatccggggggggcctggtgcagcctggggggagcctgagactgagttgtgccgcctctggggtgacatttaactactatggcatgtcttggatccgccaggcacctggaaagggcctggagtgggtggccagcatcacttcttccggcgggcgaatctactatcccgacagcgtcaagggcaggttcacaatttcccgcgagaacacacagaaaactctgtacctgcagatgaatagcctgagagccgaagatacagctgtgtactattgcactctggacggcagggatgggtgggtcgcctattgggggcagggaaccctggtgacagtcagctccggaggaggaggatctggcggaggaggcagtgggggaggcgggtcaaactttatgctgacccagccccacagtgtgtcagagagccctggcaagactgtcaccatctcttgtaaaaggaacaccggaaatattggcagtaactacgtgaattggtatcagcagcatgaagggtctagtccaaccacaatcatctaccggaacgataagagacccgacggggtgtccgatcgattctccggatctatcgaccggtcaagcaagagtgcttcactgaccattagcaatctgaaaacagaggacgaagcagattacttttgccagtcctattcctctggcttcatctttggaggcgggactaaactgaccgtgctgggcgcggccgcaggtgcaggtggtgattacaaagatgatgacgataaaggtgcagcggcgcatcaccatcatcaccac

SEQ ID NO: 80 - protein, 269 aa, Artificial Sequence
  C3E-7093 AA
GEVQLVESGGGLVQPGGSLRLSCAASGVTFNYYGMSWIRQAPGKGLEWVASITSSGGRIYYPDSVKGRFTISRENTQKTLYLQMNSLRAEDTAVYYCTLDGRDGWVAYWGQGTLVTVSSGGGGSGGGGSGGGGSNFMLTQPHSVSESPGKTVTISCKRNTGNIGSNYVNWYQQHEGSSPTTIIYRNDKRPDGVSDRFSGSIDRSSKSASLTISNLKTEDEADYFCQSYSSGFIFGGGTKLTVLGAAAGAGGDYKDDDDKGAAAHHHHHH

SEQ ID NO: 81 - DNA, 864 bp, Artificial Sequence
  C3E-7094 ORF
atgaaacacctgtggttcttcctcctgctggtggcagctcccagatgggtgctgagcggagaagtgcagctggtggaatccggggggggcctggtgcagcctggggggagcctgagactgagttgtgccgcctctggggtgacatttaactactatggcatgtcttggatccgccaggcacctggaaagggcctggagtgggtggccagcatcacttcttccggcgggcgaatctactatcccgacagcgtcaagggcaggttcacaatttcccgcgagaacacacagaaaactctgtacctgcagatgaatagcctgagagccgaagatacagctgtgtactattgcactctggacggcagggatgggtgggtcgcctattgggggcagggaaccctggtgacagtcagctccggaggaggaggatctggcggaggaggcagtgggggaggcgggtcaaactttatgctgacccagccccacagtgtgtcagagagccctggcaagactgtcaccatctcttgtaaaaggaacaccggaaatattggcagtaactacgtgaattggtatcagcagcatgaagggtctagtccaaccacaatcatctaccggagcgataagagacccgacggggtgtccgatcgattctccggatctatcgaccggtcaagcaagagtgcttcactgaccattagcaatctgaaaacagaggacgaagcagattacttttgccagtcctattcctctggcttcatctttggaggcgggactaaactgaccgtgctgggcgcggccgcaggtgcaggtggtgattacaaagatgatgacgataaaggtgcagcggcgcatcaccatcatcaccac

SEQ ID NO: 82 - protein, 269 aa, Artificial Sequence
  C3E-7094 AA
GEVQLVESGGGLVQPGGSLRLSCAASGVTFNYYGMSWIRQAPGKGLEWVASITSSGGRIYYPDSVKGRFTISRENTQKTLYLQMNSLRAEDTAVYYCTLDGRDGWVAYWGQGTLVTVSSGGGGSGGGGSGGGGSNFMLTQPHSVSESPGKTVTISCKRNTGNIGSNYVNWYQQHEGSSPTTIIYRSDKRPDGVSDRFSGSIDRSSKSASLTISNLKTEDEADYFCQSYSSGFIFGGGTKLTVLGAAAGAGGDYKDDDDKGAAAHHHHHH

SEQ ID NO: 83 - DNA, 864 bp, Artificial Sequence
  C3E-7095 ORF
atgaaacacctgtggttcttcctcctgctggtggcagctcccagatgggtgctgagcggagaagtgcagctggtggaatccggggggggcctggtgcagcctggggggagcctgagactgagttgtgccgcctctggggtgacatttaactactatggcatgtcttggatccgccaggcacctggaaagggcctggagtgggtggccagcatcacttcttccggcgggcgaatctactatcccgacagcgtcaagggcaggttcacaatttcccgcgagaacacacagaaaactctgtacctgcagatgaatagcctgagagccgaagatacagctgtgtactattgcactctggacggcagggatgggtgggtcgcctattgggggcagggaaccctggtgacagtcagctccggaggaggaggatctggcggaggaggcagtgggggaggcgggtcaaactttatgctgacccagccccacagtgtgtcagagagccctggcaagactgtcaccatctcttgtaaaaggaacaccggaaatattggcagtaactacgtgaattggtatcagcagcatgaagggtctagtccaaccacaatcatctaccgggccgataagagacccgacggggtgtccgatcgattctccggatctatcgaccggtcaagcaagagtgcttcactgaccattagcaatctgaaaacagaggacgaagcagattacttttgccagtcctattcctctggcttcatctttggaggcgggactaaactgaccgtgctgggcgcggccgcaggtgcaggtggtgattacaaagatgatgacgataaaggtgcagcggcgcatcaccatcatcaccac

SEQ ID NO: 84 - protein, 269 aa, Artificial Sequence
  C3E-7095 AA
GEVQLVESGGGLVQPGGSLRLSCAASGVTFNYYGMSWIRQAPGKGLEWVASITSSGGRIYYPDSVKGRFTISRENTQKTLYLQMNSLRAEDTAVYYCTLDGRDGWVAYWGQGTLVTVSSGGGGSGGGGSGGGGSNFMLTQPHSVSESPGKTVTISCKRNTGNIGSNYVNWYQQHEGSSPTTIIYRADKRPDGVSDRFSGSIDRSSKSASLTISNLKTEDEADYFCQSYSSGFIFGGGTKLTVLGAAAGAGGDYKDDDDKGAAAHHHHHH

SEQ ID NO: 85 - DNA, 33 bp, Artificial Sequence
  HN53R Fw
gtggccagcatcactaggtccggcgggcgaatc

SEQ ID NO: 86 - DNA, 33 bp, Artificial Sequence
  HN53R Rv
gattcgcccgccggacctagtgatgctggccac

SEQ ID NO: 87 - DNA, 33 bp, Artificial Sequence
  HN53S Fw
gtggccagcatcacttcttccggcgggcgaatc

SEQ ID NO: 88 - DNA, 33 bp, Artificial Sequence
  HN53S Rv
gattcgcccgccggaagaagtgatgctggccac

SEQ ID NO: 89 - DNA, 1590 bp, Artificial Sequence
  AXC-0001 ORF
atgaaacacctgtggttcttcctcctgctggtggcagctcccagatgggtgctgagcggagaagtgcagctgcaggaatctggccctggcctcgtgaagcctagccagaccctgagcctgacctgtaccgtgtccggctacagcatcaccagcaactactggggctggatcagaaagttccccggcaacaagatggaatggatcggccacatcaccaacagcggcaacaccacctacaaccccagcctgaagtcccggatcagcatcagccgggacaccagcaagaaccagttctccctgaagctgtccagcgtgacccctgccgataccgccgtgtactactgtgccaagggcgccttcgattactggggccagggaaccctcgtgaccgtgtctagcggaggcggaggatctggcggcggaggaagtggcggagggggatctgatatccagatgacccagagccccagcagcctgtctgccagcgtgggcgacagagtgaccatcacctgtagagccagccaggacatcggcaactacctgagctggttccagcagaaagtgggcaagtcccccagacggatgatctacggcgccatcaagctggccgtgggcgtgccaagcagattcagcggcagcagaagcggcagcgactacaccctgaccatcagctccctgcagcccgaggacttcgccatctactactgcctgcagtacatccagttccctctgaccttcggcagcggcaccaagctggaaatcaagagaaccgggggaggcggttcagaagtgcagctggtggaatccggggggggcctggtgcagcctggggggagcctgagactgagttgtgccgcctctggggtgacatttaactactatggcatgtcttggatccgccaggcacctggaaagggcctggagtgggtggccagcatcactaattccggcgggcgaatctactatcccgacagcgtcaagggcaggttcacaatttcccgcgagaacacacagaaaactctgtacctgcagatgaatagcctgagagccgaagatacagctgtgtactattgcactctggacggcagggatgggtgggtcgcctattgggggcagggaaccctggtgacagtcagctccggaggaggaggatctggcggaggaggcagtgggggaggcgggtcaaactttatgctgacccagccccacagtgtgtcagagagccctggcaagactgtcaccatctcttgtaaaaggaacaccggaaatattggcagtaactacgtgaattggtatcagcagcatgaagggtctagtccaaccacaatcatctaccgggacgataagagacccgacggggtgtccgatcgattctccggatctatcgaccggtcaagcaagagtgcttcactgaccattagcaatctgaaaacagaggacgaagcagattacttttgccagtcctattcctctggcttcatctttggaggcgggactaaactgaccgtgctgggcgcggccgcaggtgcaggtggtgattacaaagatgatgacgataaaggtgcagcggcgcatcaccatcatcaccac

SEQ ID NO: 90 - protein, 511 aa, Artificial Sequence
  AXC-0001 AA
GEVQLQESGPGLVKPSQTLSLTCTVSGYSITSNYWGWIRKFPGNKMEWIGHITNSGNTTYNPSLKSRISISRDTSKNQFSLKLSSVTPADTAVYYCAKGAFDYWGQGTLVTVSSGGGGSGGGGSGGGGSDIQMTQSPSSLSASVGDRVTITCRASQDIGNYLSWFQQKVGKSPRRMIYGAIKLAVGVPSRFSGSRSGSDYTLTISSLQPEDFAIYYCLQYIQFPLTFGSGTKLEIKRTGGGGSEVQLVESGGGLVQPGGSLRLSCAASGVTFNYYGMSWIRQAPGKGLEWVASITNSGGRIYYPDSVKGRFTISRENTQKTLYLQMNSLRAEDTAVYYCTLDGRDGWVAYWGQGTLVTVSSGGGGSGGGGSGGGGSNFMLTQPHSVSESPGKTVTISCKRNTGNIGSNYVNWYQQHEGSSPTTIIYRDDKRPDGVSDRFSGSIDRSSKSASLTISNLKTEDEADYFCQSYSSGFIFGGGTKLTVLGAAAGAGGDYKDDDDKGAAAHHHHHH

SEQ ID NO: 91 - DNA, 1584 bp, Artificial Sequence
  AXC-0002 ORF
atgaaacacctgtggttcttcctcctgctggtggcagctcccagatgggtgctgagcggagaagtgcagctgcaggaatctggccctggcctcgtgaagcctagccagaccctgagcctgacctgtaccgtgtccggctacagcatcaccagcaactactggggctggatcagaaagttccccggcaacaagatggaatggatcggccacatcaccaacagcggcaacaccacctacaaccccagcctgaagtcccggatcagcatcagccgggacaccagcaagaaccagttctccctgaagctgtccagcgtgacccctgccgataccgccgtgtactactgtgccaagggcgccttcgattactggggccagggaaccctcgtgaccgtgtctagcggaggcggaggatctggcggcggaggaagtggcggagggggatctgatatccagatgacccagagccccagcagcctgtctgccagcgtgggcgacagagtgaccatcacctgtagagccagccaggacatcggcaactacctgagctggttccagcagaaagtgggcaagtcccccagacggatgatctacggcgccatcaagctggccgtgggcgtgccaagcagattcagcggcagcagaagcggcagcgactacaccctgaccatcagctccctgcagcccgaggacttcgccatctactactgcctgcagtacatccagttccctctgaccttcggcagcggcaccaagctggaaatcaagagaaccgggggaggcggttcagaagtgcagctggtggaatccggggggggcctggtgcagcctggggggagcctgagactgagttgtgccgcctctggggtgacatttaactactatggcatgtcttggatccgccaggcacctggaaagggcctggagtgggtggccagcatcactaattccggcgggcgaatctactatcccgacagcgtcaagggcaggttcacaatttcccgcgagaacacacagaaaactctgtacctgcagatgaatagcctgagagccgaagatacagctgtgtactattgcactctggacggcagggatgggtgggtcgcctattgggggcagggaaccctggtgacagtcagctccggaggaggaggatctggcggaggaggcagtgggggaggcgggtcaaactttatgctcactcagccgtcctctgtttctggcgtacctggccaacgggtgaccattagctgtacgggtaataccgggaatatcgggtctaactacgtgaactggtatcagcagcttccagggacagctcccaagttgctgatctatcgcgacgacaaaagaccctcaggggtccctgaccgatttagtggcagcaaaagcggtacttccgcttccctggcgataaccggctttcaggccgaagatgaggcagactactattgccagtcatattccagcggcttcatcttcggaggcggaactaagctgacagtgttgggcgcggccgcaggtgcaggtggtgattacaaagatgatgacgataaaggtgcagcggcgcatcaccatcatcaccac

SEQ ID NO: 92 - protein, 509 aa, Artificial Sequence
  AXC-0002 AA
GEVQLQESGPGLVKPSQTLSLTCTVSGYSITSNYWGWIRKFPGNKMEWIGHITNSGNTTYNPSLKSRISISRDTSKNQFSLKLSSVTPADTAVYYCAKGAFDYWGQGTLVTVSSGGGGSGGGGSGGGGSDIQMTQSPSSLSASVGDRVTITCRASQDIGNYLSWFQQKVGKSPRRMIYGAIKLAVGVPSRFSGSRSGSDYTLTISSLQPEDFAIYYCLQYIQFPLTFGSGTKLEIKRTGGGGSEVQLVESGGGLVQPGGSLRLSCAASGVTFNYYGMSWIRQAPGKGLEWVASITNSGGRIYYPDSVKGRFTISRENTQKTLYLQMNSLRAEDTAVYYCTLDGRDGWVAYWGQGTLVTVSSGGGGSGGGGSGGGGSNFMLTQPSSVSGVPGQRVTISCTGNTGNIGSNYVNWYQQLPGTAPKLLIYRDDKRPSGVPDRFSGSKSGTSASLAITGFQAEDEADYYCQSYSSGFIFGGGTKLTVLGAAAGAGGDYKDDDDKGAAAHHHHHH

SEQ ID NO: 93 - DNA, 1620 bp, Artificial Sequence
  MGC-0001 ORF
atgaaacacctgtggttcttcctcctgctggtggcagctcccagatgggtgctgagcggacaggtgcagctggtgcagtctgggggaggcttggtccagcctggagggtccctgagactctcctgtgcagcctctggattcaccttcagtgactacgacatggactgggtccgccaggctccagggaaggggctggagtgggtggcagttatatcatctgatgaaaacactaaatactacgcagactccgtgaagggccgattcaccatctccagagacaattccaagaacacgctgtatctgcaaatgaacagcctgagagccgaggacacggctgtgtattactgtgcaacctataccagcacctggtatgccgttgactcctggggccagggaaccctggtcaccgtctcctcaggtggaggcggttcaggcggaggtggcagcggcggtggcgggagtgatgttgtgatgactcagtctccactctccctgcccgtcacccctggagagccggcctccatctcctgcaggtctagtcagagcctcctgcatagtaacggaaagaactatttggattggtacctgcagaagccagggcagtctccacagctcctgatctatttgggttctaatcgggcctccggggtccctgacaggttcagtggcagtggatcaggcacagattttacactgaagatcagcagagtggaggctgaggatgttggggtttattactgcatgcaaactcttcaaaccccctacacttttggccaggggaccaaggtggaaatcaaacgtgggggaggcggttcagaagtgcagctggtggaatccggggggggcctggtgcagcctggggggagcctgagactgagttgtgccgcctctggggtgacatttaactactatggcatgtcttggatccgccaggcacctggaaagggcctggagtgggtggccagcatcactaattccggcgggcgaatctactatcccgacagcgtcaagggcaggttcacaatttcccgcgagaacacacagaaaactctgtacctgcagatgaatagcctgagagccgaagatacagctgtgtactattgcactctggacggcagggatgggtgggtcgcctattgggggcagggaaccctggtgacagtcagctccggaggaggaggatctggcggaggaggcagtgggggaggcgggtcaaactttatgctgacccagccccacagtgtgtcagagagccctggcaagactgtcaccatctcttgtaaaaggaacaccggaaatattggcagtaactacgtgaattggtatcagcagcatgaagggtctagtccaaccacaatcatctaccgggacgataagagacccgacggggtgtccgatcgattctccggatctatcgaccggtcaagcaagagtgcttcactgaccattagcaatctgaaaacagaggacgaagcagattacttttgccagtcctattcctctggcttcatctttggaggcgggactaaactgaccgtgctgggcgcggccgcaggtgcaggtggtgattacaaagatgatgacgataaaggtgcagcggcgcatcaccatcatcaccac

SEQ ID NO: 94 - protein, 521 aa, Artificial Sequence
  MGC-0001 AA
GQVQLVQSGGGLVQPGGSLRLSCAASGFTFSDYDMDWVRQAPGKGLEWVAVISSDENTKYYADSVKGRFTISRDNSKNTLYLQMNSLRAEDTAVYYCATYTSTWYAVDSWGQGTLVTVSSGGGGSGGGGSGGGGSDVVMTQSPLSLPVTPGEPASISCRSSQSLLHSNGKNYLDWYLQKPGQSPQLLIYLGSNRASGVPDRFSGSGSGTDFTLKISRVEAEDVGVYYCMQTLQTPYTFGQGTKVEIKRGGGGSEVQLVESGGGLVQPGGSLRLSCAASGVTFNYYGMSWIRQAPGKGLEWVASITNSGGRIYYPDSVKGRFTISRENTQKTLYLQMNSLRAEDTAVYYCTLDGRDGWVAYWGQGTLVTVSSGGGGSGGGGSGGGGSNFMLTQPHSVSESPGKTVTISCKRNTGNIGSNYVNWYQQHEGSSPTTIIYRDDKRPDGVSDRFSGSIDRSSKSASLTISNLKTEDEADYFCQSYSSGFIFGGGTKLTVLGAAAGAGGDYKDDDDKGAAAHHHHHH

SEQ ID NO: 95 - DNA, 1614 bp, Artificial Sequence
  MGC-0002 ORF
atgaaacacctgtggttcttcctcctgctggtggcagctcccagatgggtgctgagcggacaggtgcagctggtgcagtctgggggaggcttggtccagcctggagggtccctgagactctcctgtgcagcctctggattcaccttcagtgactacgacatggactgggtccgccaggctccagggaaggggctggagtgggtggcagttatatcatctgatgaaaacactaaatactacgcagactccgtgaagggccgattcaccatctccagagacaattccaagaacacgctgtatctgcaaatgaacagcctgagagccgaggacacggctgtgtattactgtgcaacctataccagcacctggtatgccgttgactcctggggccagggaaccctggtcaccgtctcctcaggtggaggcggttcaggcggaggtggcagcggcggtggcgggagtgatgttgtgatgactcagtctccactctccctgcccgtcacccctggagagccggcctccatctcctgcaggtctagtcagagcctcctgcatagtaacggaaagaactatttggattggtacctgcagaagccagggcagtctccacagctcctgatctatttgggttctaatcgggcctccggggtccctgacaggttcagtggcagtggatcaggcacagattttacactgaagatcagcagagtggaggctgaggatgttggggtttattactgcatgcaaactcttcaaaccccctacacttttggccaggggaccaaggtggaaatcaaacgtgggggaggcggttcagaagtgcagctggtggaatccggggggggcctggtgcagcctggggggagcctgagactgagttgtgccgcctctggggtgacatttaactactatggcatgtcttggatccgccaggcacctggaaagggcctggagtgggtggccagcatcactaattccggcgggcgaatctactatcccgacagcgtcaagggcaggttcacaatttcccgcgagaacacacagaaaactctgtacctgcagatgaatagcctgagagccgaagatacagctgtgtactattgcactctggacggcagggatgggtgggtcgcctattgggggcagggaaccctggtgacagtcagctccggaggaggaggatctggcggaggaggcagtgggggaggcgggtcaaactttatgctcactcagccgtcctctgtttctggcgtacctggccaacgggtgaccattagctgtacgggtaataccgggaatatcgggtctaactacgtgaactggtatcagcagcttccagggacagctcccaagttgctgatctatcgcgacgacaaaagaccctcaggggtccctgaccgatttagtggcagcaaaagcggtacttccgcttccctggcgataaccggctttcaggccgaagatgaggcagactactattgccagtcatattccagcggcttcatcttcggaggcggaactaagctgacagtgttgggcgcggccgcaggtgcaggtggtgattacaaagatgatgacgataaaggtgcagcggcgcatcaccatcatcaccac

SEQ ID NO: 96 - protein, 519 aa, Artificial Sequence
  MGC-0002 AA
GQVQLVQSGGGLVQPGGSLRLSCAASGFTFSDYDMDWVRQAPGKGLEWVAVISSDENTKYYADSVKGRFTISRDNSKNTLYLQMNSLRAEDTAVYYCATYTSTWYAVDSWGQGTLVTVSSGGGGSGGGGSGGGGSDVVMTQSPLSLPVTPGEPASISCRSSQSLLHSNGKNYLDWYLQKPGQSPQLLIYLGSNRASGVPDRFSGSGSGTDFTLKISRVEAEDVGVYYCMQTLQTPYTFGQGTKVEIKRGGGGSEVQLVESGGGLVQPGGSLRLSCAASGVTFNYYGMSWIRQAPGKGLEWVASITNSGGRIYYPDSVKGRFTISRENTQKTLYLQMNSLRAEDTAVYYCTLDGRDGWVAYWGQGTLVTVSSGGGGSGGGGSGGGGSNFMLTQPSSVSGVPGQRVTISCTGNTGNIGSNYVNWYQQLPGTAPKLLIYRDDKRPSGVPDRFSGSKSGTSASLAITGFQAEDEADYYCQSYSSGFIFGGGTKLTVLGAAAGAGGDYKDDDDKGAAAHHHHHH

SEQ ID NO: 97 - protein, 10 aa, Homo sapiens
ILFGISLREV

SEQ ID NO: 98 - protein, 8 aa, Artificial Sequence
  CDRH2 of variants
  Xaa (3)..(3): the first Xaa is any naturally occurring amino acid
  Xaa (4)..(4): the second Xaa is any naturally occurring amino acid
ITXXGGRI

SEQ ID NO: 99 - protein, 3 aa, Artificial Sequence
  CDRL2 of variants
  X (2)..(2): Xaa is any naturally occurring amino acid
RXD

SEQ ID NO: 100 - protein, 118 aa, Artificial Sequence
  VH of C3E-7034 variants
  MISC_FEATURE (53)..(53): The first Xaa is any naturally occurring amino acid
  MISC_FEATURE (54)..(54): The second Xaa is any naturally occurring amino acid
EVQLVESGGGLVQPGGSLRLSCAASGVTFNYYGMSWIRQAPGKGLEWVASITXXGGRIYYPDSVKGRFTISRENTQKTLYLQMNSLRAEDTAVYYCTLDGRDGWVAYWGQGTLVTVSS

SEQ ID NO: 101 - protein, 109 aa, Artificial Sequence
  VL of C3E-7034 variants
  MISC_FEATURE (52)..(52): Xaa is any naturally occurring amino acid
NFMLTQPHSVSESPGKTVTISCKRNTGNIGSNYVNWYQQHEGSSPTTIIYRXDKRPDGVSDRFSGSIDRSSKSASLTISNLKTEDEADYFCQSYSSGFIFGGGTKLTVL

SEQ ID NO: 102 - protein, 107 aa, Artificial Sequence
  VL of C3E-7035 variants
  MISC_FEATURE (52)..(52): Xaa is any naturally occurring amino acid
QAVLTQPSSVSGVPGQRVTISCKRNTGNIGSNYVNWYQQLPGTAPKLLIYRXDKRPSGVPDRFSGSKSGTSASLAITGFQAEDEADYYCQSYSSGFIFGGGTKLTVL

SEQ ID NO: 103 - protein, 107 aa, Artificial Sequence
  VL of C3E-7036 variants
  MISC_FEATURE (52)..(52): Xaa is any naturally occurring amino acid
NFMLTQPSSVSGVPGQRVTISCTGNTGNIGSNYVNWYQQLPGTAPKLLIYRXDKRPSGVPDRFSGSKSGTSASLAITGFQAEDEADYYCQSYSSGFIFGGGTKLTVL